European Patent Application EP 4 431 530 A1, published September 18, 2024. Title: 用于治疗肌营养不良症的转基因表达盒. Applicant: 上海勉亦生物科技有限公司. The sequence listing filed with the application follows.

SEQUENCE LISTING (13 sequences)

SEQ ID NO: 1 - DNA, 606 bp, synthetic construct
  misc_feature 1..606: note = Nucleotide sequence of hCK promoter
  source 1..606: mol_type = other DNA
gaattcggtaccccactacgggtttaggctgcccatgtaaggaggcaaggcctggggacacccgagatgcctggttataattaacccagacatgtggctgccccccccccccccaacacctgctgcctctaaaaataaccctgtccctggtggatcccctgcatgcgaagatcttcgaacaaggctgtgggggactgagggcaggctgtaacaggcttgggggccagggcttatacgtgcctgggactcccaaagtattactgttccatgttcccggcgaagggccagctgtcccccgccagctagactcagcacttagtttaggaaccagtgagcaagtcagcccttggggcagcccatacaaggccatggggctgggcaagctgcacgcctgggtccggggtgggcacggtgcccgggcaacgagctgaaagctcatctgctctcaggggcccctccctggggacagcccctcctggctagtcacaccctgtaggctcctctatataacccaggggcacaggggctgccctcattctaccaccacctccacagcacagacagacactcaggagccagccagcgtcgagcggccgatccgccacc

SEQ ID NO: 2 - DNA, 54 bp, synthetic construct
  misc_feature 1..54: note = Nucleotide sequence of mini POLYA
  source 1..54: mol_type = other DNA
aggcctaataaagagctcagatgcatcgatcagagtgtgttggttttttgtgtg

SEQ ID NO: 3 - DNA, 8667 bp, synthetic construct
  misc_feature 1..8667: note = Nucleotide sequence of hCK-opti-M6 expression cassette
  source 1..8667: mol_type = other DNA
ctagaggtccccagcgaccttgacgagcatctgcccggcatttctgacagctttgtgaactgggtggccgagaaggaatgggagttgccgccagattctgacatggatctgaatctgattgagcaggcacccctgaccgtggccgagaagctgcatcgctggcgtaatagcgaagaggcccgcaccgatcgcccttcccaacagttgcgcagcctgaatggcgaatggcgattccgttgcaatggctggcggtaatattgttctggatattaccagcaaggccgatagtttgagttcttctactcaggcaagtgatgttattactaatcaaagaagtattgcgacaacggttaatttgcgtgatggacagactcttttactcggtggcctcactgattataaaaacacttctcaggattctggcgtaccgttcctgtctaaaatccctttaatcggcctcctgtttagctcccgctctgattctaacgaggaaagcacgttatacgtgctcgtcaaagcaaccatagtacgcgccctgtagcggcgcattaagcgcggcgggtgtggtggttacgcgcagcgtgaccgctacacttgccagcgccctagcgcccgctcctttcgctttcttcccttcctttctcgccacgttcgccggctttccccgtcaagctctaaatcgggggctccctttagggttccgatttagtgctttacggcacctcgaccccaaaaaacttgattagggtgatggttcacgtagtgggccatcgccctgatagacggtttttcgccctttgacgttggagtccacgttcttaatagtggactcttgttccaaactggaacaacactcaaccctatctcggtctattcttttgatttataagggattttgccgatttcggcctattggttaaaaaatgagctgatttaacaaaaatttaacgcgaattttaacaaaatattaacgcttacaatttaaatatttgcttatacaatcttcctgtttttggggcttttctgattatcaaccggggtacatatgattgacatgctagttttacgattaccgttcatcgcctgcaggggggggggggggggggttggccactccctctctgcgcgctcgctcgctcactgaggccgggcgaccaaaggtcgcccgacgcccgggctttgcccgggcggcctcagtgagcgagcgagcgcgcagagagggagtggccaactccatcactaggggttcctagatctgaattcggtaccccactacgggtttaggctgcccatgtaaggaggcaaggcctggggacacccgagatgcctggttataattaacccagacatgtggctgccccccccccccccaacacctgctgcctctaaaaataaccctgtccctggtggatcccctgcatgcgaagatcttcgaacaaggctgtgggggactgagggcaggctgtaacaggcttgggggccagggcttatacgtgcctgggactcccaaagtattactgttccatgttcccggcgaagggccagctgtcccccgccagctagactcagcacttagtttaggaaccagtgagcaagtcagcccttggggcagcccatacaaggccatggggctgggcaagctgcacgcctgggtccggggtgggcacggtgcccgggcaacgagctgaaagctcatctgctctcaggggcccctccctggggacagcccctcctggctagtcacaccctgtaggctcctctatataacccaggggcacaggggctgccctcattctaccaccacctccacagcacagacagacactcaggagccagccagcgtcgagcggccgatccgccaccgccaccatggccaaatatggggagcatgaggcctctccagacaatggccagaatgagttctctgacatcatcaagagcagatctgatgagcacaatgatgtgcagaagaaaaccttcaccaagtggatcaatgccaggttcagcaagtctggcaagcctcctatcaatgacatgttcacagacctgaaggatggcagaaagctgctggacctgctggaaggcctgacaggcacaagcctgcctaaagaaaggggcagcaccagagtgcatgccctgaacaatgtgaacagagtgctgcaggtcctgcaccagaacaatgttgagctggtcaatattggaggcacagacattgtggatggcaaccacaagctgaccctgggcctgctgtggtccatcatcctgcactggcaagtgaaagatgtgatgaaggatgtcatgtctgacctccagcagaccaactctgagaagatcctgctgagctgggtcagacagaccaccagaccttacagccaagtgaatgtgctgaacttcaccaccagctggacagatggcctggccttcaatgctgtgctgcacagacacaagccagacctgttcagctgggacaaagtggtcaagatgagccccattgagagactggaacatgccttcagcaaggcccagacctacctgggcattgaaaaactgctggatcctgaggatgtggcagtgcagctgcctgacaagaaatccatcatcatgtacctgaccagcctgtttgaggtgctgcctcagcaagtgaccattgatgccatcagagaggtggaaaccctgcctagaaagtacaagaaagagtgtgaagaggaagccatcaacatccagagcacagcccctgaagaggaacatgagagccccagagctgagacacccagcacagtgacagaggtggacatggacctggacagctaccagattgccctggaagaggtgctgacctggctgctgtctgctgaggacaccttccaagagcaggatgacatctctgatgatgtggaagaagtgaaggaccagtttgccacacatgaggctttcatgatggaactgacagcccaccagtcctctgtgggctctgttctgcaagctggaaaccagctgatcacccagggcaccctgagtgatgaggaagagtttgagatccaagaacagatgaccctgctgaatgccagatgggaagccctgagagtggaatccatggacagacagagcagactgcatgatgtgctcatggaactgcagaaaaagcagctgcagcaactgtctgcctggctgacactgacagaagaaaggatccagaagatggaaacctgtccactggatgatgatgttaagagcctgcagaagctcctggaagaacacaagtccctgcagtctgacctggaagctgagcaagtcaaagtgaacagcctgacacacatggtggtcatagtggatgagaactctggggagtctgccacagccattctggaagatcagctccagaaactgggagaaagatggacagctgtgtgcagatggactgaggaaaggtggaacagactgcaagagatcaatatcctgtggcaagagctgcttgaggaacagtgcctgctgaaagcttggctgactgagaaagaagaggctctgaacaaggtgcagaccagcaacttcaaggaccagaaagaactgtctgtgtctgtcagaaggctggccatcctgaaagaggacatggaaatgaagagacagaccctggaccagctgtctgagattggccaggatgtgggccagcttctggacaactctaaggccagcaagaagatcaactctgactctgaggaactgacccagagatgggactccctggtgcagaggctggaagatagcagcaatcaagtgacccaggctgtggccaagctgggcatgtctcagatccctcagaaggatctgctggaaacagttagagttagagagcaggccatcaccaagaagtccaagcaagaactggaagccagctctgaccagtggaagaggctgcacctgagcctccaagaactgcttgtgtggctgcagctcaaggatgatgagctgagcagacaggcccctattggtggagacttccctgctgtgcagaaacagaatgatgtccacagggccttcaagagggaactcaagaccaaagaacctgtgatcatgagcaccctggaaactgtcagaatcttcctgactgagcagcccctggaaggactggaaaagctgtaccaagagcctagagagctgcctcctgaagaaagggcccagaatgtgacaagactgctgagaaagcaggctgaggaagtgaacactgagtgggagaagctgaatctgcactctgctgactggcagagaaagatagatgagacactggaaaggctccaagagttgcaagaggccacagatgagctggatctgaaactgagacaggctgaagtgatcaaaggcagctggcagcctgtgggagatctgctgattgacagcctgcaggaccacctggaaaaagtcaaggccctgaggggagagattgcccctctgaaagaaaatgtgtcccatgtgaatgacctggccagacagctcaccacactgggcattcaactgagcccctacaacctgtctacccttgaggacctgaacaccagatggaagctgctccaggtggcagttgaggacagagttagacagctgcatgaggctcacagagactttggccctgccagccagcacttcctgagcacctctgtgcaaggcccttgggagagagctatcagccccaacaaagtgccctactacatcaaccatgagactcagaccacctgttgggatcaccccaagatgacagagctgtatcagagcctggcagacctcaacaatgtcagattcagtgcctacaggacagccatgaagctgagaaggctccagaaggccctctgcctggatctcctgtctctgtctgcagcttgtgatgccctggatcagcacaacctgaagcagaatgatcagcccatggacatcctgcagatcatcaactgcctgaccacaatctatgacaggctggaacaagagcacaacaacctggtcaatgtgcccctgtgtgtggacatgtgcctgaattggctgctcaatgtgtatgacacaggcaggacaggcagaatcagggtgctgagcttcaagacaggcatcatcagcctgtgcaaagctcacttggaggacaagtacagatacctgttcaaacaggtggccagcagcacaggcttttgtgaccagagaaggcttggcctgctgctgcatgacagcattcagatccccaggcagcttggagaggtggcctcctttggaggcagcaatattgagccctctgtcaggtcctgtttccaatttgccaacaacaagcctgagattgaggctgccctgttcctggactggatgagacttgagccccagtccatggtctggctgccagtgctgcatagagtggctgctgcagagacagccaagcaccaggccaaatgcaacatctgcaaagagtgccccatcattggcttcagatacagaagcctgaagcacttcaactatgatatctgccagagctgtttctttagtggcagagtggccaagggccacaagatgcactaccccatggtggaatactgcacccctaccacctctggggaagatgttagagattttgccaaggtgctgaagaacaagttcaggaccaagagatactttgctaagcaccccaggatgggctatctgcctgtgcagacagtgcttgagggagacaacatggaaacatgatgaggagctcgagaggcctaataaagagctcagatgcatcgatcagagtgtgttggttttttgtgtgagatctaggaacccctagtgatggagttggccactccctctctgcgcgctcgctcgctcactgaggccgcccgggcaaagcccgggcgtcgggcgacctttggtcgcccggcctcagtgagcgagcgagcgcgcagagagggagtggccaacccccccccccccccccctgcaggcgattctcttgtttgctccagactctcaggcaatgacctgatagcctttgtagagacctctcaaaaatagctaccctctccggcatgaatttatcagctagaacggttgaatatcatattgatggtgatttgactgtctccggcctttctcacccgtttgaatctttacctacacattactcaggcattgcatttaaaatatatgagggttctaaaaatttttatccttgcgttgaaataaaggcttctcccgcaaaagtattacagggtcataatgtttttggtacaaccgatttagctttatgctctgaggctttattgcttaattttgctaattctttgccttgcctgtatgatttattggatgttggaatcgcctgatgcggtattttctccttacgcatctgtgcggtatttcacaccgcatatggtgcactctcagtacaatctgctctgatgccgcatagttaagccagccccgacacccgccaacacccgctgacgcgccctgacgggcttgtctgctcccggcatccgcttacagacaagctgtgaccgtctccgggagctgcatgtgtcagaggttttcaccgtcatcaccgaaacgcgcgagacgaaagggcctcgtgatacgcctatttttataggttaatgtcatgataataatggtttcttagacgtcaggtggcacttttcggggaaatgtgcgcggaacccctatttgtttatttttctaaatacattcaaatatgtatccgctcatgagacaataaccctgataaatgcttcaataatattgaaaaaggaagagtatgattgaacaagatggattgcacgcaggttctccggccgcttgggtggagaggctattcggctatgactgggcacaacagacaatcggctgctctgatgccgccgtgttccggctgtcagcgcaggggcgcccggttctttttgtcaagaccgacctgtccggtgccctgaatgaactgcaagacgaggcagcgcggctatcgtggctggccacgacgggcgttccttgcgcagctgtgctcgatgttgtcactgaagcgggaagggactggctgctattgggcgaagtgccggggcaggatctcctgtcatctcaccttgctcctgccgagaaagtatccatcatggctgatgcaatgcggcggctgcatacgcttgatccggctacctgcccattcgaccaccaagcgaaacatcgcatcgagcgagcacgtactcggatggaagccggtcttgtcgatcaggatgatctggacgaagagcatcaggggctcgcgccagccgaactgttcgccaggctcaaggcgagcatgcccgacggcgaggatctcgtcgtgacccatggcgatgcctgcttgccgaatatcatggtggaaaatggccgcttttctggattcatcgactgtggccggctgggtgtggcggaccgctatcaggacatagcgttggctacccgtgatattgctgaagagcttggcggcgaatgggctgaccgcttcctcgtgctttacggtatcgccgctcccgattcgcagcgcatcgccttctatcgccttcttgacgagttcttctgactgtcagaccaagtttactcatatatactttagattgatttaaaacttcatttttaatttaaaaggatctaggtgaagatcctttttgataatctcatgaccaaaatcccttaacgtgagttttcgttccactgagcgtcagaccccgtagaaaagatcaaaggatcttcttgagatcctttttttctgcgcgtaatctgctgcttgcaaacaaaaaaaccaccgctaccagcggtggtttgtttgccggatcaagagctaccaactctttttccgaaggtaactggcttcagcagagcgcagataccaaatactgttcttctagtgtagccgtagttaggccaccacttcaagaactctgtagcaccgcctacatacctcgctctgctaatcctgttaccagtggctgctgccagtggcgataagtcgtgtcttaccgggttggactcaagacgatagttaccggataaggcgcagcggtcgggctgaacggggggttcgtgcacacagcccagcttggagcgaacgacctacaccgaactgagatacctacagcgtgagctatgagaaagcgccacgcttcccgaagggagaaaggcggacaggtatccggtaagcggcagggtcggaacaggagagcgcacgagggagcttccagggggaaacgcctggtatctttatagtcctgtcgggtttcgccacctctgacttgagcgtcgatttttgtgatgctcgtcaggggggcggagcctatggaaaaacgccagcaacgcggcctttttacggttcctggccttttgctggccttttgctcacatgttctttcctgcgttatcccctgattctgtggataaccgtattaccgcctttgagtgagctgataccgctcgccgcagccgaacgaccgagcgcagcgagtcagtgagcgaggaagcggaagagcgcccaatacgcaaaccgcctctccccgcgcgttggccgattcattaatgcagaattcccatcatcaataatataccttattttggattgaagccaatatgataatgagggggtggagtttgtgacgtggcgcggggcgtgggaacggggcgggtgacgtagtagct

SEQ ID NO: 4 - protein, 1279 aa, synthetic construct
  REGION 1..1279: note = Amino acid sequence of recombinant fusion protein (protein product of M6 or opti-M6 construct)
MAKYGEHEASPDNGQNEFSDIIKSRSDEHNDVQKKTFTKWINARFSKSGKPPINDMFTDLKDGRKLLDLLEGLTGTSLPKERGSTRVHALNNVNRVLQVLHQNNVELVNIGGTDIVDGNHKLTLGLLWSIILHWQVKDVMKDVMSDLQQTNSEKILLSWVRQTTRPYSQVNVLNFTTSWTDGLAFNAVLHRHKPDLFSWDKVVKMSPIERLEHAFSKAQTYLGIEKLLDPEDVAVQLPDKKSIIMYLTSLFEVLPQQVTIDAIREVETLPRKYKKECEEEAINIQSTAPEEEHESPRAETPSTVTEVDMDLDSYQIALEEVLTWLLSAEDTFQEQDDISDDVEEVKDQFATHEAFMMELTAHQSSVGSVLQAGNQLITQGTLSDEEEFEIQEQMTLLNARWEALRVESMDRQSRLHDVLMELQKKQLQQLSAWLTLTEERIQKMETCPLDDDVKSLQKLLEEHKSLQSDLEAEQVKVNSLTHMVVIVDENSGESATAILEDQLQKLGERWTAVCRWTEERWNRLQEINILWQELLEEQCLLKAWLTEKEEALNKVQTSNFKDQKELSVSVRRLAILKEDMEMKRQTLDQLSEIGQDVGQLLDNSKASKKINSDSEELTQRWDSLVQRLEDSSNQVTQAVAKLGMSQIPQKDLLETVRVREQAITKKSKQELEASSDQWKRLHLSLQELLVWLQLKDDELSRQAPIGGDFPAVQKQNDVHRAFKRELKTKEPVIMSTLETVRIFLTEQPLEGLEKLYQEPRELPPEERAQNVTRLLRKQAEEVNTEWEKLNLHSADWQRKIDETLERLQELQEATDELDLKLRQAEVIKGSWQPVGDLLIDSLQDHLEKVKALRGEIAPLKENVSHVNDLARQLTTLGIQLSPYNLSTLEDLNTRWKLLQVAVEDRVRQLHEAHRDFGPASQHFLSTSVQGPWERAISPNKVPYYINHETQTTCWDHPKMTELYQSLADLNNVRFSAYRTAMKLRRLQKALCLDLLSLSAACDALDQHNLKQNDQPMDILQIINCLTTIYDRLEQEHNNLVNVPLCVDMCLNWLLNVYDTGRTGRIRVLSFKTGIISLCKAHLEDKYRYLFKQVASSTGFCDQRRLGLLLHDSIQIPRQLGEVASFGGSNIEPSVRSCFQFANNKPEIEAALFLDWMRLEPQSMVWLPVLHRVAAAETAKHQAKCNICKECPIIGFRYRSLKHFNYDICQSCFFSGRVAKGHKMHYPMVEYCTPTTSGEDVRDFAKVLKNKFRTKRYFAKHPRMGYLPVQTVLEGDNMET

SEQ ID NO: 5 - DNA, 8667 bp, synthetic construct
  misc_feature 1..8667: note = Nucleotide sequence of hCK-M6 expression cassette
  source 1..8667: mol_type = other DNA
ctagaggtccccagcgaccttgacgagcatctgcccggcatttctgacagctttgtgaactgggtggccgagaaggaatgggagttgccgccagattctgacatggatctgaatctgattgagcaggcacccctgaccgtggccgagaagctgcatcgctggcgtaatagcgaagaggcccgcaccgatcgcccttcccaacagttgcgcagcctgaatggcgaatggcgattccgttgcaatggctggcggtaatattgttctggatattaccagcaaggccgatagtttgagttcttctactcaggcaagtgatgttattactaatcaaagaagtattgcgacaacggttaatttgcgtgatggacagactcttttactcggtggcctcactgattataaaaacacttctcaggattctggcgtaccgttcctgtctaaaatccctttaatcggcctcctgtttagctcccgctctgattctaacgaggaaagcacgttatacgtgctcgtcaaagcaaccatagtacgcgccctgtagcggcgcattaagcgcggcgggtgtggtggttacgcgcagcgtgaccgctacacttgccagcgccctagcgcccgctcctttcgctttcttcccttcctttctcgccacgttcgccggctttccccgtcaagctctaaatcgggggctccctttagggttccgatttagtgctttacggcacctcgaccccaaaaaacttgattagggtgatggttcacgtagtgggccatcgccctgatagacggtttttcgccctttgacgttggagtccacgttcttaatagtggactcttgttccaaactggaacaacactcaaccctatctcggtctattcttttgatttataagggattttgccgatttcggcctattggttaaaaaatgagctgatttaacaaaaatttaacgcgaattttaacaaaatattaacgcttacaatttaaatatttgcttatacaatcttcctgtttttggggcttttctgattatcaaccggggtacatatgattgacatgctagttttacgattaccgttcatcgcctgcaggggggggggggggggggttggccactccctctctgcgcgctcgctcgctcactgaggccgggcgaccaaaggtcgcccgacgcccgggctttgcccgggcggcctcagtgagcgagcgagcgcgcagagagggagtggccaactccatcactaggggttcctagatctgaattcggtaccccactacgggtttaggctgcccatgtaaggaggcaaggcctggggacacccgagatgcctggttataattaacccagacatgtggctgccccccccccccccaacacctgctgcctctaaaaataaccctgtccctggtggatcccctgcatgcgaagatcttcgaacaaggctgtgggggactgagggcaggctgtaacaggcttgggggccagggcttatacgtgcctgggactcccaaagtattactgttccatgttcccggcgaagggccagctgtcccccgccagctagactcagcacttagtttaggaaccagtgagcaagtcagcccttggggcagcccatacaaggccatggggctgggcaagctgcacgcctgggtccggggtgggcacggtgcccgggcaacgagctgaaagctcatctgctctcaggggcccctccctggggacagcccctcctggctagtcacaccctgtaggctcctctatataacccaggggcacaggggctgccctcattctaccaccacctccacagcacagacagacactcaggagccagccagcgtcgagcggccgatccgccaccgccaccatggccaaatatggcgagcatgaggctagccccgacaacggccagaacgagttcagcgacatcatcaagagcagaagcgacgagcacaacgacgtgcagaagaaaaccttcaccaagtggatcaacgcccggttcagcaagagcggcaagcctcctatcaacgacatgttcaccgacctgaaggacggcagaaagctgctggatctgctggaaggcctgaccggcacaagcctgcctaaagaaaggggcagcacaagagtgcacgccctgaacaacgtgaaccgggtgctgcaggttctgcaccagaacaatgtggaactggtcaacatcggcggcaccgacatcgtggacggcaatcacaaactgaccctgggcctgctgtggtccatcatcctgcactggcaagtgaaagacgtgatgaaggatgtgatgagcgatctgcagcagaccaacagcgagaagatcctgctgagctgggtccgacagaccaccagaccttacagccaagtgaacgtgctgaacttcaccaccagctggacagacggcctggcctttaatgccgtgctgcacagacacaagcccgacctgttcagctgggacaaagtggtcaagatgagccccatcgagcggctggaacacgccttttctaaggcccagacctacctgggcatcgaaaaactgctggaccccgaggatgtggccgtgcagctgcctgacaagaaatccatcatcatgtacctgaccagcctgttcgaggtgctgcctcagcaagtgaccatcgacgccatcagagaggtggaaaccctgcctcggaagtacaagaaagagtgcgaggaagaggccatcaacatccagagcacagcccctgaggaagaacacgagagccctagagccgagacacctagcacagtgaccgaggtggacatggacctggacagctatcagatcgccctggaagaggtgctgacctggctgctgtctgccgaggataccttccaagagcaggacgacatcagcgacgacgtggaagaagtgaaggaccagttcgccacacacgaggccttcatgatggaactgacagcccaccagtctagcgtgggctctgttctgcaagccggcaaccagctgatcacccagggcaccctgtctgatgaggaagagttcgagatccaagaacagatgaccctgctgaacgccagatgggaagccctgagagtggaatccatggaccggcagagcagactgcacgacgtgctcatggaactgcagaaaaagcagctgcagcagctcagcgcctggctgacactgaccgaagaacggatccagaagatggaaacctgtcctctggacgacgatgtgaagtccctgcagaagctgctcgaggaacacaagagcctgcagagcgacctggaagccgagcaagtcaaagtgaacagcctgacacacatggtcgtgatcgtggatgagaacagcggcgagtctgccacagccatcctggaagatcagctgcagaaactgggcgagagatggaccgccgtgtgcagatggacagaggaacggtggaaccggctgcaagagatcaatatcctgtggcaagaactcctcgaagaacagtgtctgctgaaggcttggctgaccgagaaagaagaggctctgaacaaggtgcagaccagcaacttcaaggaccagaaagaactgagcgtgtccgtgcggagactggccattctgaaagaggacatggaaatgaagcggcagaccctggaccagctgtctgagatcggacaggatgtgggccagctcctggacaatagcaaggccagcaagaagatcaacagcgacagcgaggaactgacccagagatgggattcactggtgcagcggctcgaggacagcagcaatcaagtgacacaggccgtggccaagctgggcatgtctcagatccctcagaaggacctgctggaaaccgtcagagtcagagagcaggccatcaccaagaagtccaagcaagaactggaagccagctccgaccagtggaagagactgcacctgtctctgcaagagctgctcgtgtggctgcagctcaaggacgatgagctgagcagacaggcccctatcggcggagattttcccgccgtgcagaaacagaacgatgtgcaccgggccttcaagcgcgagctgaaaacaaaagaacccgtgatcatgagcaccctggaaacagtgcggatcttcctgaccgagcagcccctggaaggactggaaaagctgtaccaagagcctagagagctgcctcctgaagaacgggcccagaacgtgaccagactgctgagaaagcaggccgaggaagtgaacaccgagtgggagaagctgaacctgcacagcgccgactggcagcggaagattgacgagacactggaaagactccaagaactgcaagaggccaccgacgagctggacctgaaactgagacaggccgaagtgatcaaaggcagctggcagcctgtgggcgacctgctgattgatagcctgcaggaccacctcgagaaagtgaaggctctgagaggcgagatcgcccctctgaaagaaaacgtgtcccacgtgaacgacctggctcggcagctgacaacactgggaattcagctgagcccctacaacctgtccacactcgaggacctgaacacccggtggaaactgcttcaggtggccgtggaagatagagtgcgccagctgcatgaggcccacagagattttggacctgccagccagcacttcctgagcacctctgtgcaaggcccttgggagagagctatcagccccaacaaagtgccctactacatcaaccacgagacacagaccacatgctgggatcaccccaagatgaccgagctgtatcagagcctggccgacctcaacaacgtgcggtttagcgcctaccggaccgccatgaagctgcggaggctgcaaaaagccctgtgcctggatctcctgagcctgagcgctgcttgtgatgccctggatcagcacaatctgaagcagaacgaccagcctatggacatcctgcagatcatcaactgcctgaccaccatctacgaccgcctggaacaagagcacaacaacctggtcaacgtgcccctgtgcgtggacatgtgcctgaattggctgctgaatgtgtacgacaccggcagaaccggcaggatcagagtgctgagcttcaagaccggcatcatcagcctgtgcaaagcccaccttgaggacaagtaccgctacctgttcaaacaggtggccagcagcaccggcttttgcgaccaaagaaggctgggactgctgctgcacgacagcattcagatcccacggcagctgggagaagtggccagctttggcggcagcaatatcgagcctagcgtgcggtcctgctttcagtttgccaacaacaagcctgagatcgaggccgctctgttcctggactggatgagactggaaccccagagcatggtctggctgcctgtgctgcatagagtggctgccgccgaaacagccaagcaccaggccaagtgcaacatctgcaaagagtgccccatcatcggcttccggtacagaagcctgaagcacttcaactacgatatctgccagtcctgcttcttcagcggcagagtggccaagggccacaagatgcactaccccatggtggaatactgcacccctaccaccagcggagaggacgtgcgggattttgccaaggtgctgaagaacaagttccggaccaagcgctacttcgctaagcaccccagaatgggctatctgcccgtgcagacagtcctggaaggcgacaacatggaaacctgatgaggagctcgagaggcctaataaagagctcagatgcatcgatcagagtgtgttggttttttgtgtgagatctaggaacccctagtgatggagttggccactccctctctgcgcgctcgctcgctcactgaggccgcccgggcaaagcccgggcgtcgggcgacctttggtcgcccggcctcagtgagcgagcgagcgcgcagagagggagtggccaacccccccccccccccccctgcaggcgattctcttgtttgctccagactctcaggcaatgacctgatagcctttgtagagacctctcaaaaatagctaccctctccggcatgaatttatcagctagaacggttgaatatcatattgatggtgatttgactgtctccggcctttctcacccgtttgaatctttacctacacattactcaggcattgcatttaaaatatatgagggttctaaaaatttttatccttgcgttgaaataaaggcttctcccgcaaaagtattacagggtcataatgtttttggtacaaccgatttagctttatgctctgaggctttattgcttaattttgctaattctttgccttgcctgtatgatttattggatgttggaatcgcctgatgcggtattttctccttacgcatctgtgcggtatttcacaccgcatatggtgcactctcagtacaatctgctctgatgccgcatagttaagccagccccgacacccgccaacacccgctgacgcgccctgacgggcttgtctgctcccggcatccgcttacagacaagctgtgaccgtctccgggagctgcatgtgtcagaggttttcaccgtcatcaccgaaacgcgcgagacgaaagggcctcgtgatacgcctatttttataggttaatgtcatgataataatggtttcttagacgtcaggtggcacttttcggggaaatgtgcgcggaacccctatttgtttatttttctaaatacattcaaatatgtatccgctcatgagacaataaccctgataaatgcttcaataatattgaaaaaggaagagtatgattgaacaagatggattgcacgcaggttctccggccgcttgggtggagaggctattcggctatgactgggcacaacagacaatcggctgctctgatgccgccgtgttccggctgtcagcgcaggggcgcccggttctttttgtcaagaccgacctgtccggtgccctgaatgaactgcaagacgaggcagcgcggctatcgtggctggccacgacgggcgttccttgcgcagctgtgctcgatgttgtcactgaagcgggaagggactggctgctattgggcgaagtgccggggcaggatctcctgtcatctcaccttgctcctgccgagaaagtatccatcatggctgatgcaatgcggcggctgcatacgcttgatccggctacctgcccattcgaccaccaagcgaaacatcgcatcgagcgagcacgtactcggatggaagccggtcttgtcgatcaggatgatctggacgaagagcatcaggggctcgcgccagccgaactgttcgccaggctcaaggcgagcatgcccgacggcgaggatctcgtcgtgacccatggcgatgcctgcttgccgaatatcatggtggaaaatggccgcttttctggattcatcgactgtggccggctgggtgtggcggaccgctatcaggacatagcgttggctacccgtgatattgctgaagagcttggcggcgaatgggctgaccgcttcctcgtgctttacggtatcgccgctcccgattcgcagcgcatcgccttctatcgccttcttgacgagttcttctgactgtcagaccaagtttactcatatatactttagattgatttaaaacttcatttttaatttaaaaggatctaggtgaagatcctttttgataatctcatgaccaaaatcccttaacgtgagttttcgttccactgagcgtcagaccccgtagaaaagatcaaaggatcttcttgagatcctttttttctgcgcgtaatctgctgcttgcaaacaaaaaaaccaccgctaccagcggtggtttgtttgccggatcaagagctaccaactctttttccgaaggtaactggcttcagcagagcgcagataccaaatactgttcttctagtgtagccgtagttaggccaccacttcaagaactctgtagcaccgcctacatacctcgctctgctaatcctgttaccagtggctgctgccagtggcgataagtcgtgtcttaccgggttggactcaagacgatagttaccggataaggcgcagcggtcgggctgaacggggggttcgtgcacacagcccagcttggagcgaacgacctacaccgaactgagatacctacagcgtgagctatgagaaagcgccacgcttcccgaagggagaaaggcggacaggtatccggtaagcggcagggtcggaacaggagagcgcacgagggagcttccagggggaaacgcctggtatctttatagtcctgtcgggtttcgccacctctgacttgagcgtcgatttttgtgatgctcgtcaggggggcggagcctatggaaaaacgccagcaacgcggcctttttacggttcctggccttttgctggccttttgctcacatgttctttcctgcgttatcccctgattctgtggataaccgtattaccgcctttgagtgagctgataccgctcgccgcagccgaacgaccgagcgcagcgagtcagtgagcgaggaagcggaagagcgcccaatacgcaaaccgcctctccccgcgcgttggccgattcattaatgcagaattcccatcatcaataatataccttattttggattgaagccaatatgataatgagggggtggagtttgtgacgtggcgcggggcgtgggaacggggcgggtgacgtagtagct

SEQ ID NO: 6 - DNA, 8641 bp, synthetic construct
  misc_feature 1..8641: note = Nucleotide sequence of shCK-opti-M6 expression cassette
  source 1..8641: mol_type = other DNA
ctagaggtccccagcgaccttgacgagcatctgcccggcatttctgacagctttgtgaactgggtggccgagaaggaatgggagttgccgccagattctgacatggatctgaatctgattgagcaggcacccctgaccgtggccgagaagctgcatcgctggcgtaatagcgaagaggcccgcaccgatcgcccttcccaacagttgcgcagcctgaatggcgaatggcgattccgttgcaatggctggcggtaatattgttctggatattaccagcaaggccgatagtttgagttcttctactcaggcaagtgatgttattactaatcaaagaagtattgcgacaacggttaatttgcgtgatggacagactcttttactcggtggcctcactgattataaaaacacttctcaggattctggcgtaccgttcctgtctaaaatccctttaatcggcctcctgtttagctcccgctctgattctaacgaggaaagcacgttatacgtgctcgtcaaagcaaccatagtacgcgccctgtagcggcgcattaagcgcggcgggtgtggtggttacgcgcagcgtgaccgctacacttgccagcgccctagcgcccgctcctttcgctttcttcccttcctttctcgccacgttcgccggctttccccgtcaagctctaaatcgggggctccctttagggttccgatttagtgctttacggcacctcgaccccaaaaaacttgattagggtgatggttcacgtagtgggccatcgccctgatagacggtttttcgccctttgacgttggagtccacgttcttaatagtggactcttgttccaaactggaacaacactcaaccctatctcggtctattcttttgatttataagggattttgccgatttcggcctattggttaaaaaatgagctgatttaacaaaaatttaacgcgaattttaacaaaatattaacgcttacaatttaaatatttgcttatacaatcttcctgtttttggggcttttctgattatcaaccggggtacatatgattgacatgctagttttacgattaccgttcatcgcctgcaggggggggggggggggggttggccactccctctctgcgcgctcgctcgctcactgaggccgggcgaccaaaggtcgcccgacgcccgggctttgcccgggcggcctcagtgagcgagcgagcgcgcagagagggagtggccaactccatcactaggggttcctagatctgaattcggtaccccactacgggtttaggctgcccatgtaaggaggcaaggcctggggacacccgagatgcctggttataattaacccagacatgtggctgccccccccccccccaacacctgctgcctctaaaaataaccctgtccctggtggatcccctgcatgcgaagatcttcgaacaaggctgtgggggactgagggcaggctgtaacaggcttgggggccagggcttatacgtgcctgggactcccaaagtattactgttccatgttcccggcgaagggccagctgtcccccgccagctagactcagcacttagtttaggaaccagtgagcaagtcagcccttggggcagcccatacaaggccatggggctgggcaagctgcacgcctgggtccggggtgggcacggtgcccgggcaacgagctgaaagctcatctgctctcaggggcccctccctggggacagcccctcctggctagtcacaccctgtaggctcctctatataacccaggggcacaggggctgccctcattctaccaccaccacagcacagacagacaaaactcctaaaaaaccgccaccatggccaaatatggggagcatgaggcctctccagacaatggccagaatgagttctctgacatcatcaagagcagatctgatgagcacaatgatgtgcagaagaaaaccttcaccaagtggatcaatgccaggttcagcaagtctggcaagcctcctatcaatgacatgttcacagacctgaaggatggcagaaagctgctggacctgctggaaggcctgacaggcacaagcctgcctaaagaaaggggcagcaccagagtgcatgccctgaacaatgtgaacagagtgctgcaggtcctgcaccagaacaatgttgagctggtcaatattggaggcacagacattgtggatggcaaccacaagctgaccctgggcctgctgtggtccatcatcctgcactggcaagtgaaagatgtgatgaaggatgtcatgtctgacctccagcagaccaactctgagaagatcctgctgagctgggtcagacagaccaccagaccttacagccaagtgaatgtgctgaacttcaccaccagctggacagatggcctggccttcaatgctgtgctgcacagacacaagccagacctgttcagctgggacaaagtggtcaagatgagccccattgagagactggaacatgccttcagcaaggcccagacctacctgggcattgaaaaactgctggatcctgaggatgtggcagtgcagctgcctgacaagaaatccatcatcatgtacctgaccagcctgtttgaggtgctgcctcagcaagtgaccattgatgccatcagagaggtggaaaccctgcctagaaagtacaagaaagagtgtgaagaggaagccatcaacatccagagcacagcccctgaagaggaacatgagagccccagagctgagacacccagcacagtgacagaggtggacatggacctggacagctaccagattgccctggaagaggtgctgacctggctgctgtctgctgaggacaccttccaagagcaggatgacatctctgatgatgtggaagaagtgaaggaccagtttgccacacatgaggctttcatgatggaactgacagcccaccagtcctctgtgggctctgttctgcaagctggaaaccagctgatcacccagggcaccctgagtgatgaggaagagtttgagatccaagaacagatgaccctgctgaatgccagatgggaagccctgagagtggaatccatggacagacagagcagactgcatgatgtgctcatggaactgcagaaaaagcagctgcagcaactgtctgcctggctgacactgacagaagaaaggatccagaagatggaaacctgtccactggatgatgatgttaagagcctgcagaagctcctggaagaacacaagtccctgcagtctgacctggaagctgagcaagtcaaagtgaacagcctgacacacatggtggtcatagtggatgagaactctggggagtctgccacagccattctggaagatcagctccagaaactgggagaaagatggacagctgtgtgcagatggactgaggaaaggtggaacagactgcaagagatcaatatcctgtggcaagagctgcttgaggaacagtgcctgctgaaagcttggctgactgagaaagaagaggctctgaacaaggtgcagaccagcaacttcaaggaccagaaagaactgtctgtgtctgtcagaaggctggccatcctgaaagaggacatggaaatgaagagacagaccctggaccagctgtctgagattggccaggatgtgggccagcttctggacaactctaaggccagcaagaagatcaactctgactctgaggaactgacccagagatgggactccctggtgcagaggctggaagatagcagcaatcaagtgacccaggctgtggccaagctgggcatgtctcagatccctcagaaggatctgctggaaacagttagagttagagagcaggccatcaccaagaagtccaagcaagaactggaagccagctctgaccagtggaagaggctgcacctgagcctccaagaactgcttgtgtggctgcagctcaaggatgatgagctgagcagacaggcccctattggtggagacttccctgctgtgcagaaacagaatgatgtccacagggccttcaagagggaactcaagaccaaagaacctgtgatcatgagcaccctggaaactgtcagaatcttcctgactgagcagcccctggaaggactggaaaagctgtaccaagagcctagagagctgcctcctgaagaaagggcccagaatgtgacaagactgctgagaaagcaggctgaggaagtgaacactgagtgggagaagctgaatctgcactctgctgactggcagagaaagatagatgagacactggaaaggctccaagagttgcaagaggccacagatgagctggatctgaaactgagacaggctgaagtgatcaaaggcagctggcagcctgtgggagatctgctgattgacagcctgcaggaccacctggaaaaagtcaaggccctgaggggagagattgcccctctgaaagaaaatgtgtcccatgtgaatgacctggccagacagctcaccacactgggcattcaactgagcccctacaacctgtctacccttgaggacctgaacaccagatggaagctgctccaggtggcagttgaggacagagttagacagctgcatgaggctcacagagactttggccctgccagccagcacttcctgagcacctctgtgcaaggcccttgggagagagctatcagccccaacaaagtgccctactacatcaaccatgagactcagaccacctgttgggatcaccccaagatgacagagctgtatcagagcctggcagacctcaacaatgtcagattcagtgcctacaggacagccatgaagctgagaaggctccagaaggccctctgcctggatctcctgtctctgtctgcagcttgtgatgccctggatcagcacaacctgaagcagaatgatcagcccatggacatcctgcagatcatcaactgcctgaccacaatctatgacaggctggaacaagagcacaacaacctggtcaatgtgcccctgtgtgtggacatgtgcctgaattggctgctcaatgtgtatgacacaggcaggacaggcagaatcagggtgctgagcttcaagacaggcatcatcagcctgtgcaaagctcacttggaggacaagtacagatacctgttcaaacaggtggccagcagcacaggcttttgtgaccagagaaggcttggcctgctgctgcatgacagcattcagatccccaggcagcttggagaggtggcctcctttggaggcagcaatattgagccctctgtcaggtcctgtttccaatttgccaacaacaagcctgagattgaggctgccctgttcctggactggatgagacttgagccccagtccatggtctggctgccagtgctgcatagagtggctgctgcagagacagccaagcaccaggccaaatgcaacatctgcaaagagtgccccatcattggcttcagatacagaagcctgaagcacttcaactatgatatctgccagagctgtttctttagtggcagagtggccaagggccacaagatgcactaccccatggtggaatactgcacccctaccacctctggggaagatgttagagattttgccaaggtgctgaagaacaagttcaggaccaagagatactttgctaagcaccccaggatgggctatctgcctgtgcagacagtgcttgagggagacaacatggaaacatgatgaggagctcgagaggcctaataaagagctcagatgcatcgatcagagtgtgttggttttttgtgtgagatctaggaacccctagtgatggagttggccactccctctctgcgcgctcgctcgctcactgaggccgcccgggcaaagcccgggcgtcgggcgacctttggtcgcccggcctcagtgagcgagcgagcgcgcagagagggagtggccaacccccccccccccccccctgcaggcgattctcttgtttgctccagactctcaggcaatgacctgatagcctttgtagagacctctcaaaaatagctaccctctccggcatgaatttatcagctagaacggttgaatatcatattgatggtgatttgactgtctccggcctttctcacccgtttgaatctttacctacacattactcaggcattgcatttaaaatatatgagggttctaaaaatttttatccttgcgttgaaataaaggcttctcccgcaaaagtattacagggtcataatgtttttggtacaaccgatttagctttatgctctgaggctttattgcttaattttgctaattctttgccttgcctgtatgatttattggatgttggaatcgcctgatgcggtattttctccttacgcatctgtgcggtatttcacaccgcatatggtgcactctcagtacaatctgctctgatgccgcatagttaagccagccccgacacccgccaacacccgctgacgcgccctgacgggcttgtctgctcccggcatccgcttacagacaagctgtgaccgtctccgggagctgcatgtgtcagaggttttcaccgtcatcaccgaaacgcgcgagacgaaagggcctcgtgatacgcctatttttataggttaatgtcatgataataatggtttcttagacgtcaggtggcacttttcggggaaatgtgcgcggaacccctatttgtttatttttctaaatacattcaaatatgtatccgctcatgagacaataaccctgataaatgcttcaataatattgaaaaaggaagagtatgattgaacaagatggattgcacgcaggttctccggccgcttgggtggagaggctattcggctatgactgggcacaacagacaatcggctgctctgatgccgccgtgttccggctgtcagcgcaggggcgcccggttctttttgtcaagaccgacctgtccggtgccctgaatgaactgcaagacgaggcagcgcggctatcgtggctggccacgacgggcgttccttgcgcagctgtgctcgatgttgtcactgaagcgggaagggactggctgctattgggcgaagtgccggggcaggatctcctgtcatctcaccttgctcctgccgagaaagtatccatcatggctgatgcaatgcggcggctgcatacgcttgatccggctacctgcccattcgaccaccaagcgaaacatcgcatcgagcgagcacgtactcggatggaagccggtcttgtcgatcaggatgatctggacgaagagcatcaggggctcgcgccagccgaactgttcgccaggctcaaggcgagcatgcccgacggcgaggatctcgtcgtgacccatggcgatgcctgcttgccgaatatcatggtggaaaatggccgcttttctggattcatcgactgtggccggctgggtgtggcggaccgctatcaggacatagcgttggctacccgtgatattgctgaagagcttggcggcgaatgggctgaccgcttcctcgtgctttacggtatcgccgctcccgattcgcagcgcatcgccttctatcgccttcttgacgagttcttctgactgtcagaccaagtttactcatatatactttagattgatttaaaacttcatttttaatttaaaaggatctaggtgaagatcctttttgataatctcatgaccaaaatcccttaacgtgagttttcgttccactgagcgtcagaccccgtagaaaagatcaaaggatcttcttgagatcctttttttctgcgcgtaatctgctgcttgcaaacaaaaaaaccaccgctaccagcggtggtttgtttgccggatcaagagctaccaactctttttccgaaggtaactggcttcagcagagcgcagataccaaatactgttcttctagtgtagccgtagttaggccaccacttcaagaactctgtagcaccgcctacatacctcgctctgctaatcctgttaccagtggctgctgccagtggcgataagtcgtgtcttaccgggttggactcaagacgatagttaccggataaggcgcagcggtcgggctgaacggggggttcgtgcacacagcccagcttggagcgaacgacctacaccgaactgagatacctacagcgtgagctatgagaaagcgccacgcttcccgaagggagaaaggcggacaggtatccggtaagcggcagggtcggaacaggagagcgcacgagggagcttccagggggaaacgcctggtatctttatagtcctgtcgggtttcgccacctctgacttgagcgtcgatttttgtgatgctcgtcaggggggcggagcctatggaaaaacgccagcaacgcggcctttttacggttcctggccttttgctggccttttgctcacatgttctttcctgcgttatcccctgattctgtggataaccgtattaccgcctttgagtgagctgataccgctcgccgcagccgaacgaccgagcgcagcgagtcagtgagcgaggaagcggaagagcgcccaatacgcaaaccgcctctccccgcgcgttggccgattcattaatgcagaattcccatcatcaataatataccttattttggattgaagccaatatgataatgagggggtggagtttgtgacgtggcgcggggcgtgggaacggggcgggtgacgtagtagct

SEQ ID NO: 7 - DNA, 8641 bp, synthetic construct
  misc_feature 1..8641: note = Nucleotide sequence of shCK-M6 expression cassette
  source 1..8641: mol_type = other DNA
ctagaggtccccagcgaccttgacgagcatctgcccggcatttctgacagctttgtgaactgggtggccgagaaggaatgggagttgccgccagattctgacatggatctgaatctgattgagcaggcacccctgaccgtggccgagaagctgcatcgctggcgtaatagcgaagaggcccgcaccgatcgcccttcccaacagttgcgcagcctgaatggcgaatggcgattccgttgcaatggctggcggtaatattgttctggatattaccagcaaggccgatagtttgagttcttctactcaggcaagtgatgttattactaatcaaagaagtattgcgacaacggttaatttgcgtgatggacagactcttttactcggtggcctcactgattataaaaacacttctcaggattctggcgtaccgttcctgtctaaaatccctttaatcggcctcctgtttagctcccgctctgattctaacgaggaaagcacgttatacgtgctcgtcaaagcaaccatagtacgcgccctgtagcggcgcattaagcgcggcgggtgtggtggttacgcgcagcgtgaccgctacacttgccagcgccctagcgcccgctcctttcgctttcttcccttcctttctcgccacgttcgccggctttccccgtcaagctctaaatcgggggctccctttagggttccgatttagtgctttacggcacctcgaccccaaaaaacttgattagggtgatggttcacgtagtgggccatcgccctgatagacggtttttcgccctttgacgttggagtccacgttcttaatagtggactcttgttccaaactggaacaacactcaaccctatctcggtctattcttttgatttataagggattttgccgatttcggcctattggttaaaaaatgagctgatttaacaaaaatttaacgcgaattttaacaaaatattaacgcttacaatttaaatatttgcttatacaatcttcctgtttttggggcttttctgattatcaaccggggtacatatgattgacatgctagttttacgattaccgttcatcgcctgcaggggggggggggggggggttggccactccctctctgcgcgctcgctcgctcactgaggccgggcgaccaaaggtcgcccgacgcccgggctttgcccgggcggcctcagtgagcgagcgagcgcgcagagagggagtggccaactccatcactaggggttcctagatctgaattcggtaccccactacgggtttaggctgcccatgtaaggaggcaaggcctggggacacccgagatgcctggttataattaacccagacatgtggctgccccccccccccccaacacctgctgcctctaaaaataaccctgtccctggtggatcccctgcatgcgaagatcttcgaacaaggctgtgggggactgagggcaggctgtaacaggcttgggggccagggcttatacgtgcctgggactcccaaagtattactgttccatgttcccggcgaagggccagctgtcccccgccagctagactcagcacttagtttaggaaccagtgagcaagtcagcccttggggcagcccatacaaggccatggggctgggcaagctgcacgcctgggtccggggtgggcacggtgcccgggcaacgagctgaaagctcatctgctctcaggggcccctccctggggacagcccctcctggctagtcacaccctgtaggctcctctatataacccaggggcacaggggctgccctcattctaccaccaccacagcacagacagacaaaactcctaaaaaaccgccaccatggccaaatatggcgagcatgaggctagccccgacaacggccagaacgagttcagcgacatcatcaagagcagaagcgacgagcacaacgacgtgcagaagaaaaccttcaccaagtggatcaacgcccggttcagcaagagcggcaagcctcctatcaacgacatgttcaccgacctgaaggacggcagaaagctgctggatctgctggaaggcctgaccggcacaagcctgcctaaagaaaggggcagcacaagagtgcacgccctgaacaacgtgaaccgggtgctgcaggttctgcaccagaacaatgtggaactggtcaacatcggcggcaccgacatcgtggacggcaatcacaaactgaccctgggcctgctgtggtccatcatcctgcactggcaagtgaaagacgtgatgaaggatgtgatgagcgatctgcagcagaccaacagcgagaagatcctgctgagctgggtccgacagaccaccagaccttacagccaagtgaacgtgctgaacttcaccaccagctggacagacggcctggcctttaatgccgtgctgcacagacacaagcccgacctgttcagctgggacaaagtggtcaagatgagccccatcgagcggctggaacacgccttttctaaggcccagacctacctgggcatcgaaaaactgctggaccccgaggatgtggccgtgcagctgcctgacaagaaatccatcatcatgtacctgaccagcctgttcgaggtgctgcctcagcaagtgaccatcgacgccatcagagaggtggaaaccctgcctcggaagtacaagaaagagtgcgaggaagaggccatcaacatccagagcacagcccctgaggaagaacacgagagccctagagccgagacacctagcacagtgaccgaggtggacatggacctggacagctatcagatcgccctggaagaggtgctgacctggctgctgtctgccgaggataccttccaagagcaggacgacatcagcgacgacgtggaagaagtgaaggaccagttcgccacacacgaggccttcatgatggaactgacagcccaccagtctagcgtgggctctgttctgcaagccggcaaccagctgatcacccagggcaccctgtctgatgaggaagagttcgagatccaagaacagatgaccctgctgaacgccagatgggaagccctgagagtggaatccatggaccggcagagcagactgcacgacgtgctcatggaactgcagaaaaagcagctgcagcagctcagcgcctggctgacactgaccgaagaacggatccagaagatggaaacctgtcctctggacgacgatgtgaagtccctgcagaagctgctcgaggaacacaagagcctgcagagcgacctggaagccgagcaagtcaaagtgaacagcctgacacacatggtcgtgatcgtggatgagaacagcggcgagtctgccacagccatcctggaagatcagctgcagaaactgggcgagagatggaccgccgtgtgcagatggacagaggaacggtggaaccggctgcaagagatcaatatcctgtggcaagaactcctcgaagaacagtgtctgctgaaggcttggctgaccgagaaagaagaggctctgaacaaggtgcagaccagcaacttcaaggaccagaaagaactgagcgtgtccgtgcggagactggccattctgaaagaggacatggaaatgaagcggcagaccctggaccagctgtctgagatcggacaggatgtgggccagctcctggacaatagcaaggccagcaagaagatcaacagcgacagcgaggaactgacccagagatgggattcactggtgcagcggctcgaggacagcagcaatcaagtgacacaggccgtggccaagctgggcatgtctcagatccctcagaaggacctgctggaaaccgtcagagtcagagagcaggccatcaccaagaagtccaagcaagaactggaagccagctccgaccagtggaagagactgcacctgtctctgcaagagctgctcgtgtggctgcagctcaaggacgatgagctgagcagacaggcccctatcggcggagattttcccgccgtgcagaaacagaacgatgtgcaccgggccttcaagcgcgagctgaaaacaaaagaacccgtgatcatgagcaccctggaaacagtgcggatcttcctgaccgagcagcccctggaaggactggaaaagctgtaccaagagcctagagagctgcctcctgaagaacgggcccagaacgtgaccagactgctgagaaagcaggccgaggaagtgaacaccgagtgggagaagctgaacctgcacagcgccgactggcagcggaagattgacgagacactggaaagactccaagaactgcaagaggccaccgacgagctggacctgaaactgagacaggccgaagtgatcaaaggcagctggcagcctgtgggcgacctgctgattgatagcctgcaggaccacctcgagaaagtgaaggctctgagaggcgagatcgcccctctgaaagaaaacgtgtcccacgtgaacgacctggctcggcagctgacaacactgggaattcagctgagcccctacaacctgtccacactcgaggacctgaacacccggtggaaactgcttcaggtggccgtggaagatagagtgcgccagctgcatgaggcccacagagattttggacctgccagccagcacttcctgagcacctctgtgcaaggcccttgggagagagctatcagccccaacaaagtgccctactacatcaaccacgagacacagaccacatgctgggatcaccccaagatgaccgagctgtatcagagcctggccgacctcaacaacgtgcggtttagcgcctaccggaccgccatgaagctgcggaggctgcaaaaagccctgtgcctggatctcctgagcctgagcgctgcttgtgatgccctggatcagcacaatctgaagcagaacgaccagcctatggacatcctgcagatcatcaactgcctgaccaccatctacgaccgcctggaacaagagcacaacaacctggtcaacgtgcccctgtgcgtggacatgtgcctgaattggctgctgaatgtgtacgacaccggcagaaccggcaggatcagagtgctgagcttcaagaccggcatcatcagcctgtgcaaagcccaccttgaggacaagtaccgctacctgttcaaacaggtggccagcagcaccggcttttgcgaccaaagaaggctgggactgctgctgcacgacagcattcagatcccacggcagctgggagaagtggccagctttggcggcagcaatatcgagcctagcgtgcggtcctgctttcagtttgccaacaacaagcctgagatcgaggccgctctgttcctggactggatgagactggaaccccagagcatggtctggctgcctgtgctgcatagagtggctgccgccgaaacagccaagcaccaggccaagtgcaacatctgcaaagagtgccccatcatcggcttccggtacagaagcctgaagcacttcaactacgatatctgccagtcctgcttcttcagcggcagagtggccaagggccacaagatgcactaccccatggtggaatactgcacccctaccaccagcggagaggacgtgcgggattttgccaaggtgctgaagaacaagttccggaccaagcgctacttcgctaagcaccccagaatgggctatctgcccgtgcagacagtcctggaaggcgacaacatggaaacctgatgaggagctcgagaggcctaataaagagctcagatgcatcgatcagagtgtgttggttttttgtgtgagatctaggaacccctagtgatggagttggccactccctctctgcgcgctcgctcgctcactgaggccgcccgggcaaagcccgggcgtcgggcgacctttggtcgcccggcctcagtgagcgagcgagcgcgcagagagggagtggccaacccccccccccccccccctgcaggcgattctcttgtttgctccagactctcaggcaatgacctgatagcctttgtagagacctctcaaaaatagctaccctctccggcatgaatttatcagctagaacggttgaatatcatattgatggtgatttgactgtctccggcctttctcacccgtttgaatctttacctacacattactcaggcattgcatttaaaatatatgagggttctaaaaatttttatccttgcgttgaaataaaggcttctcccgcaaaagtattacagggtcataatgtttttggtacaaccgatttagctttatgctctgaggctttattgcttaattttgctaattctttgccttgcctgtatgatttattggatgttggaatcgcctgatgcggtattttctccttacgcatctgtgcggtatttcacaccgcatatggtgcactctcagtacaatctgctctgatgccgcatagttaagccagccccgacacccgccaacacccgctgacgcgccctgacgggcttgtctgctcccggcatccgcttacagacaagctgtgaccgtctccgggagctgcatgtgtcagaggttttcaccgtcatcaccgaaacgcgcgagacgaaagggcctcgtgatacgcctatttttataggttaatgtcatgataataatggtttcttagacgtcaggtggcacttttcggggaaatgtgcgcggaacccctatttgtttatttttctaaatacattcaaatatgtatccgctcatgagacaataaccctgataaatgcttcaataatattgaaaaaggaagagtatgattgaacaagatggattgcacgcaggttctccggccgcttgggtggagaggctattcggctatgactgggcacaacagacaatcggctgctctgatgccgccgtgttccggctgtcagcgcaggggcgcccggttctttttgtcaagaccgacctgtccggtgccctgaatgaactgcaagacgaggcagcgcggctatcgtggctggccacgacgggcgttccttgcgcagctgtgctcgatgttgtcactgaagcgggaagggactggctgctattgggcgaagtgccggggcaggatctcctgtcatctcaccttgctcctgccgagaaagtatccatcatggctgatgcaatgcggcggctgcatacgcttgatccggctacctgcccattcgaccaccaagcgaaacatcgcatcgagcgagcacgtactcggatggaagccggtcttgtcgatcaggatgatctggacgaagagcatcaggggctcgcgccagccgaactgttcgccaggctcaaggcgagcatgcccgacggcgaggatctcgtcgtgacccatggcgatgcctgcttgccgaatatcatggtggaaaatggccgcttttctggattcatcgactgtggccggctgggtgtggcggaccgctatcaggacatagcgttggctacccgtgatattgctgaagagcttggcggcgaatgggctgaccgcttcctcgtgctttacggtatcgccgctcccgattcgcagcgcatcgccttctatcgccttcttgacgagttcttctgactgtcagaccaagtttactcatatatactttagattgatttaaaacttcatttttaatttaaaaggatctaggtgaagatcctttttgataatctcatgaccaaaatcccttaacgtgagttttcgttccactgagcgtcagaccccgtagaaaagatcaaaggatcttcttgagatcctttttttctgcgcgtaatctgctgcttgcaaacaaaaaaaccaccgctaccagcggtggtttgtttgccggatcaagagctaccaactctttttccgaaggtaactggcttcagcagagcgcagataccaaatactgttcttctagtgtagccgtagttaggccaccacttcaagaactctgtagcaccgcctacatacctcgctctgctaatcctgttaccagtggctgctgccagtggcgataagtcgtgtcttaccgggttggactcaagacgatagttaccggataaggcgcagcggtcgggctgaacggggggttcgtgcacacagcccagcttggagcgaacgacctacaccgaactgagatacctacagcgtgagctatgagaaagcgccacgcttcccgaagggagaaaggcggacaggtatccggtaagcggcagggtcggaacaggagagcgcacgagggagcttccagggggaaacgcctggtatctttatagtcctgtcgggtttcgccacctctgacttgagcgtcgatttttgtgatgctcgtcaggggggcggagcctatggaaaaacgccagcaacgcggcctttttacggttcctggccttttgctggccttttgctcacatgttctttcctgcgttatcccctgattctgtggataaccgtattaccgcctttgagtgagctgataccgctcgccgcagccgaacgaccgagcgcagcgagtcagtgagcgaggaagcggaagagcgcccaatacgcaaaccgcctctccccgcgcgttggccgattcattaatgcagaattcccatcatcaataatataccttattttggattgaagccaatatgataatgagggggtggagtttgtgacgtggcgcggggcgtgggaacggggcgggtgacgtagtagct

SEQ ID NO: 8 - DNA, 3840 bp, synthetic construct
  misc_feature 1..3840: note = Nucleotide sequence of opti-M6 construct
  source 1..3840: mol_type = other DNA
atggccaaatatggggagcatgaggcctctccagacaatggccagaatgagttctctgacatcatcaagagcagatctgatgagcacaatgatgtgcagaagaaaaccttcaccaagtggatcaatgccaggttcagcaagtctggcaagcctcctatcaatgacatgttcacagacctgaaggatggcagaaagctgctggacctgctggaaggcctgacaggcacaagcctgcctaaagaaaggggcagcaccagagtgcatgccctgaacaatgtgaacagagtgctgcaggtcctgcaccagaacaatgttgagctggtcaatattggaggcacagacattgtggatggcaaccacaagctgaccctgggcctgctgtggtccatcatcctgcactggcaagtgaaagatgtgatgaaggatgtcatgtctgacctccagcagaccaactctgagaagatcctgctgagctgggtcagacagaccaccagaccttacagccaagtgaatgtgctgaacttcaccaccagctggacagatggcctggccttcaatgctgtgctgcacagacacaagccagacctgttcagctgggacaaagtggtcaagatgagccccattgagagactggaacatgccttcagcaaggcccagacctacctgggcattgaaaaactgctggatcctgaggatgtggcagtgcagctgcctgacaagaaatccatcatcatgtacctgaccagcctgtttgaggtgctgcctcagcaagtgaccattgatgccatcagagaggtggaaaccctgcctagaaagtacaagaaagagtgtgaagaggaagccatcaacatccagagcacagcccctgaagaggaacatgagagccccagagctgagacacccagcacagtgacagaggtggacatggacctggacagctaccagattgccctggaagaggtgctgacctggctgctgtctgctgaggacaccttccaagagcaggatgacatctctgatgatgtggaagaagtgaaggaccagtttgccacacatgaggctttcatgatggaactgacagcccaccagtcctctgtgggctctgttctgcaagctggaaaccagctgatcacccagggcaccctgagtgatgaggaagagtttgagatccaagaacagatgaccctgctgaatgccagatgggaagccctgagagtggaatccatggacagacagagcagactgcatgatgtgctcatggaactgcagaaaaagcagctgcagcaactgtctgcctggctgacactgacagaagaaaggatccagaagatggaaacctgtccactggatgatgatgttaagagcctgcagaagctcctggaagaacacaagtccctgcagtctgacctggaagctgagcaagtcaaagtgaacagcctgacacacatggtggtcatagtggatgagaactctggggagtctgccacagccattctggaagatcagctccagaaactgggagaaagatggacagctgtgtgcagatggactgaggaaaggtggaacagactgcaagagatcaatatcctgtggcaagagctgcttgaggaacagtgcctgctgaaagcttggctgactgagaaagaagaggctctgaacaaggtgcagaccagcaacttcaaggaccagaaagaactgtctgtgtctgtcagaaggctggccatcctgaaagaggacatggaaatgaagagacagaccctggaccagctgtctgagattggccaggatgtgggccagcttctggacaactctaaggccagcaagaagatcaactctgactctgaggaactgacccagagatgggactccctggtgcagaggctggaagatagcagcaatcaagtgacccaggctgtggccaagctgggcatgtctcagatccctcagaaggatctgctggaaacagttagagttagagagcaggccatcaccaagaagtccaagcaagaactggaagccagctctgaccagtggaagaggctgcacctgagcctccaagaactgcttgtgtggctgcagctcaaggatgatgagctgagcagacaggcccctattggtggagacttccctgctgtgcagaaacagaatgatgtccacagggccttcaagagggaactcaagaccaaagaacctgtgatcatgagcaccctggaaactgtcagaatcttcctgactgagcagcccctggaaggactggaaaagctgtaccaagagcctagagagctgcctcctgaagaaagggcccagaatgtgacaagactgctgagaaagcaggctgaggaagtgaacactgagtgggagaagctgaatctgcactctgctgactggcagagaaagatagatgagacactggaaaggctccaagagttgcaagaggccacagatgagctggatctgaaactgagacaggctgaagtgatcaaaggcagctggcagcctgtgggagatctgctgattgacagcctgcaggaccacctggaaaaagtcaaggccctgaggggagagattgcccctctgaaagaaaatgtgtcccatgtgaatgacctggccagacagctcaccacactgggcattcaactgagcccctacaacctgtctacccttgaggacctgaacaccagatggaagctgctccaggtggcagttgaggacagagttagacagctgcatgaggctcacagagactttggccctgccagccagcacttcctgagcacctctgtgcaaggcccttgggagagagctatcagccccaacaaagtgccctactacatcaaccatgagactcagaccacctgttgggatcaccccaagatgacagagctgtatcagagcctggcagacctcaacaatgtcagattcagtgcctacaggacagccatgaagctgagaaggctccagaaggccctctgcctggatctcctgtctctgtctgcagcttgtgatgccctggatcagcacaacctgaagcagaatgatcagcccatggacatcctgcagatcatcaactgcctgaccacaatctatgacaggctggaacaagagcacaacaacctggtcaatgtgcccctgtgtgtggacatgtgcctgaattggctgctcaatgtgtatgacacaggcaggacaggcagaatcagggtgctgagcttcaagacaggcatcatcagcctgtgcaaagctcacttggaggacaagtacagatacctgttcaaacaggtggccagcagcacaggcttttgtgaccagagaaggcttggcctgctgctgcatgacagcattcagatccccaggcagcttggagaggtggcctcctttggaggcagcaatattgagccctctgtcaggtcctgtttccaatttgccaacaacaagcctgagattgaggctgccctgttcctggactggatgagacttgagccccagtccatggtctggctgccagtgctgcatagagtggctgctgcagagacagccaagcaccaggccaaatgcaacatctgcaaagagtgccccatcattggcttcagatacagaagcctgaagcacttcaactatgatatctgccagagctgtttctttagtggcagagtggccaagggccacaagatgcactaccccatggtggaatactgcacccctaccacctctggggaagatgttagagattttgccaaggtgctgaagaacaagttcaggaccaagagatactttgctaagcaccccaggatgggctatctgcctgtgcagacagtgcttgagggagacaacatggaaacatga

SEQ ID NO: 9 - DNA, 580 bp, synthetic construct
  misc_feature 1..580: note = Nucleotide sequence of shCK promoter
  source 1..580: mol_type = other DNA
gaattcggtaccccactacgggtttaggctgcccatgtaaggaggcaaggcctggggacacccgagatgcctggttataattaacccagacatgtggctgccccccccccccccaacacctgctgcctctaaaaataaccctgtccctggtggatcccctgcatgcgaagatcttcgaacaaggctgtgggggactgagggcaggctgtaacaggcttgggggccagggcttatacgtgcctgggactcccaaagtattactgttccatgttcccggcgaagggccagctgtcccccgccagctagactcagcacttagtttaggaaccagtgagcaagtcagcccttggggcagcccatacaaggccatggggctgggcaagctgcacgcctgggtccggggtgggcacggtgcccgggcaacgagctgaaagctcatctgctctcaggggcccctccctggggacagcccctcctggctagtcacaccctgtaggctcctctatataacccaggggcacaggggctgccctcattctaccaccaccacagcacagacagacaaaactcctaaaaaacc

SEQ ID NO: 10 - DNA, 3840 bp, synthetic construct
  misc_feature 1..3840: note = Nucleotide sequence of M6 construct
  source 1..3840: mol_type = other DNA
atggccaaatatggcgagcatgaggctagccccgacaacggccagaacgagttcagcgacatcatcaagagcagaagcgacgagcacaacgacgtgcagaagaaaaccttcaccaagtggatcaacgcccggttcagcaagagcggcaagcctcctatcaacgacatgttcaccgacctgaaggacggcagaaagctgctggatctgctggaaggcctgaccggcacaagcctgcctaaagaaaggggcagcacaagagtgcacgccctgaacaacgtgaaccgggtgctgcaggttctgcaccagaacaatgtggaactggtcaacatcggcggcaccgacatcgtggacggcaatcacaaactgaccctgggcctgctgtggtccatcatcctgcactggcaagtgaaagacgtgatgaaggatgtgatgagcgatctgcagcagaccaacagcgagaagatcctgctgagctgggtccgacagaccaccagaccttacagccaagtgaacgtgctgaacttcaccaccagctggacagacggcctggcctttaatgccgtgctgcacagacacaagcccgacctgttcagctgggacaaagtggtcaagatgagccccatcgagcggctggaacacgccttttctaaggcccagacctacctgggcatcgaaaaactgctggaccccgaggatgtggccgtgcagctgcctgacaagaaatccatcatcatgtacctgaccagcctgttcgaggtgctgcctcagcaagtgaccatcgacgccatcagagaggtggaaaccctgcctcggaagtacaagaaagagtgcgaggaagaggccatcaacatccagagcacagcccctgaggaagaacacgagagccctagagccgagacacctagcacagtgaccgaggtggacatggacctggacagctatcagatcgccctggaagaggtgctgacctggctgctgtctgccgaggataccttccaagagcaggacgacatcagcgacgacgtggaagaagtgaaggaccagttcgccacacacgaggccttcatgatggaactgacagcccaccagtctagcgtgggctctgttctgcaagccggcaaccagctgatcacccagggcaccctgtctgatgaggaagagttcgagatccaagaacagatgaccctgctgaacgccagatgggaagccctgagagtggaatccatggaccggcagagcagactgcacgacgtgctcatggaactgcagaaaaagcagctgcagcagctcagcgcctggctgacactgaccgaagaacggatccagaagatggaaacctgtcctctggacgacgatgtgaagtccctgcagaagctgctcgaggaacacaagagcctgcagagcgacctggaagccgagcaagtcaaagtgaacagcctgacacacatggtcgtgatcgtggatgagaacagcggcgagtctgccacagccatcctggaagatcagctgcagaaactgggcgagagatggaccgccgtgtgcagatggacagaggaacggtggaaccggctgcaagagatcaatatcctgtggcaagaactcctcgaagaacagtgtctgctgaaggcttggctgaccgagaaagaagaggctctgaacaaggtgcagaccagcaacttcaaggaccagaaagaactgagcgtgtccgtgcggagactggccattctgaaagaggacatggaaatgaagcggcagaccctggaccagctgtctgagatcggacaggatgtgggccagctcctggacaatagcaaggccagcaagaagatcaacagcgacagcgaggaactgacccagagatgggattcactggtgcagcggctcgaggacagcagcaatcaagtgacacaggccgtggccaagctgggcatgtctcagatccctcagaaggacctgctggaaaccgtcagagtcagagagcaggccatcaccaagaagtccaagcaagaactggaagccagctccgaccagtggaagagactgcacctgtctctgcaagagctgctcgtgtggctgcagctcaaggacgatgagctgagcagacaggcccctatcggcggagattttcccgccgtgcagaaacagaacgatgtgcaccgggccttcaagcgcgagctgaaaacaaaagaacccgtgatcatgagcaccctggaaacagtgcggatcttcctgaccgagcagcccctggaaggactggaaaagctgtaccaagagcctagagagctgcctcctgaagaacgggcccagaacgtgaccagactgctgagaaagcaggccgaggaagtgaacaccgagtgggagaagctgaacctgcacagcgccgactggcagcggaagattgacgagacactggaaagactccaagaactgcaagaggccaccgacgagctggacctgaaactgagacaggccgaagtgatcaaaggcagctggcagcctgtgggcgacctgctgattgatagcctgcaggaccacctcgagaaagtgaaggctctgagaggcgagatcgcccctctgaaagaaaacgtgtcccacgtgaacgacctggctcggcagctgacaacactgggaattcagctgagcccctacaacctgtccacactcgaggacctgaacacccggtggaaactgcttcaggtggccgtggaagatagagtgcgccagctgcatgaggcccacagagattttggacctgccagccagcacttcctgagcacctctgtgcaaggcccttgggagagagctatcagccccaacaaagtgccctactacatcaaccacgagacacagaccacatgctgggatcaccccaagatgaccgagctgtatcagagcctggccgacctcaacaacgtgcggtttagcgcctaccggaccgccatgaagctgcggaggctgcaaaaagccctgtgcctggatctcctgagcctgagcgctgcttgtgatgccctggatcagcacaatctgaagcagaacgaccagcctatggacatcctgcagatcatcaactgcctgaccaccatctacgaccgcctggaacaagagcacaacaacctggtcaacgtgcccctgtgcgtggacatgtgcctgaattggctgctgaatgtgtacgacaccggcagaaccggcaggatcagagtgctgagcttcaagaccggcatcatcagcctgtgcaaagcccaccttgaggacaagtaccgctacctgttcaaacaggtggccagcagcaccggcttttgcgaccaaagaaggctgggactgctgctgcacgacagcattcagatcccacggcagctgggagaagtggccagctttggcggcagcaatatcgagcctagcgtgcggtcctgctttcagtttgccaacaacaagcctgagatcgaggccgctctgttcctggactggatgagactggaaccccagagcatggtctggctgcctgtgctgcatagagtggctgccgccgaaacagccaagcaccaggccaagtgcaacatctgcaaagagtgccccatcatcggcttccggtacagaagcctgaagcacttcaactacgatatctgccagtcctgcttcttcagcggcagagtggccaagggccacaagatgcactaccccatggtggaatactgcacccctaccaccagcggagaggacgtgcgggattttgccaaggtgctgaagaacaagttccggaccaagcgctacttcgctaagcaccccagaatgggctatctgcccgtgcagacagtcctggaaggcgacaacatggaaacctga

SEQ ID NO: 11 - DNA, 3978 bp, synthetic construct
  misc_feature 1..3978: note = Nucleotide sequence of B84
  source 1..3978: mol_type = other DNA
atgctttggtgggaggaagtggaggactgctacgagagagaggacgtgcagaagaaaaccttcaccaagtgggtgaacgcccagttcagcaagttcggcaagcagcacatcgagaacctgttcagcgacctgcaggatggcaggagactgctggacctgctggagggcctgaccggccagaagctgcccaaggagaagggcagcaccagagtgcacgccctgaacaacgtgaacaaggccctgagagtgctgcagaacaacaacgtggacctggtgaacatcggcagcaccgacatcgtggacggcaaccacaagctgaccctgggcctgatctggaacatcatcctgcactggcaggtgaagaacgtgatgaagaacatcatggccggcctgcagcagaccaacagcgagaagatcctgctgagctgggtgaggcagagcaccagaaactacccccaggtgaacgtgatcaacttcaccacctcctggagcgacggcctggccctgaacgccctgatccacagccacagacccgacctgttcgactggaacagcgtggtgtgtcagcagagcgccacccagagactggagcacgccttcaacatcgccagataccagctgggcatcgagaagctgctggaccccgaggacgtggacaccacctaccccgacaagaaaagcatcctcatgtacattaccagcctgttccaggtgctgccccagcaggtgtccatcgaggccatccaggaagtggaaatgctgcccaggccccccaaagtgaccaaggaggagcacttccagctgcaccaccagatgcactacagccagcagatcacagtgagcctggcccagggctatgagagaaccagcagccccaagcccagattcaagagctacgcctacacccaggccgcctacgtgaccacctccgaccccaccagaagccccttccccagccagcacctggaggcccccgaggacaagagcttcggcagcagcctgatggagagcgaagtgaacctggacagataccagaccgccctggaggaagtgctgtcctggctgctgagcgccgaggacaccctgcaggcccagggcgagatcagcaacgacgtggaagtggtgaaggaccagttccacacccacgagggctacatgatggatctgaccgcccaccagggcagagtgggcaatatcctgcagctgggcagcaagctgatcggcaccggcaagctgagcgaggacgaggagaccgaagtgcaggagcagatgaacctgctgaacagcagatgggagtgcctgagagtggccagcatggagaagcagagcaacctgcacagagtgctgatggacctgcagaaccagaagctgaaggagctgaacgactggctgaccaagaccgaggagcggaccagaaagatggaggaggagcccctgggccccgacctggaggacctgaagagacaggtgcagcagcacaaagtgctgcaggaggacctggagcaggagcaggtgcgcgtgaacagcctgacccacatggtggtggtcgtggacgagagcagcggcgaccacgccacagccgccctggaagagcagctgaaagtgctgggcgacagatgggccaatatttgtaggtggaccgaggacagatgggtgctgctgcaggaccagcccgacctggcccctggcctgaccaccatcggcgccagccccacccagaccgtgaccctggtgacccagcccgtggtgacaaaggagaccgccatcagcaagctggagatgcccagctccctgatgctggaagtgcccacccaccgcctgctccagcagttccccctggacctggagaagttcctggcctggctgaccgaggccgaaaccaccgccaatgtgctccaggacgccactagaaaggagaggctgctggaggacagcaagggcgtgaaagagctgatgaagcagtggcaggatctgcagggcgaaatcgaggcccacaccgacgtgtaccacaacctggacgagaacagccagaagattctgaggagcctggagggcagcgacgacgccgtcctgctccagaggaggctggacaacatgaacttcaagtggagcgagctgcggaagaagagcctgaacatccggagccacctggaagccagcagcgaccagtggaagagactgcacctgagcctgcaggagctgctggtgtggctgcagctgaaggacgacgagctgagcagacaggcccccatcggcggcgacttccccgccgtgcagaagcagaacgacgtgcaccgggccttcaagagggagctgaaaaccaaggaacccgtgatcatgagcaccctggagacagtgcggatcttcctgaccgagcagcccctggagggactggagaagctgtaccaggagcccagagagctgccccccgaggagagagcccagaacgtgaccaggctgctgagaaagcaggccgaggaagtgaataccgagtgggagaagctgaatctgcacagcgccgactggcagagaaagatcgacgagaccctggagagactccaggaactgcaggaagccaccgacgagctggacctgaagctgagacaggccgaagtgatcaagggcagctggcagcctgtgggcgatctgctgatcgactccctgcaggatcacctggagaaagtgaaggccctgcggggcgagatcgcccccctgaaggagaatgtgagccacgtgaacgacctggccagacagctgaccaccctgggcatccagctgagcccctacaacctgagcacactggaggatctgaacacccggtggaaactgctgcaggtggccgtggaggatagagtgaggcagctgcacgaagcccacagagacttcggccctgcctcccagcacttcctgagcaccagcgtgcagggcccctgggagagagccatctcccccaacaaagtgccctactacatcaaccacgagacccagaccacctgctgggaccaccctaagatgaccgagctgtatcagagcctggccgacctgaacaatgtgcggttcagcgcctacagaaccgccatgaagctgcggagactgcagaaggccctgtgcctggatctgctgagcctgagcgccgcctgcgacgccctggaccagcacaacctgaagcagaatgaccagcccatggacatcctgcagatcatcaactgcctgaccacaatctacgaccggctggaacaggagcacaacaacctggtgaatgtgcccctgtgcgtggacatgtgcctgaattggctgctgaacgtgtacgacaccggcaggaccggcagaatccgcgtgctgagcttcaagaccggcatcatcagcctgtgcaaggcccacctggaggataagtaccgctacctgttcaagcaggtggccagcagcaccggcttctgcgatcagaggagactgggcctgctgctgcacgatagcatccagatccctaggcagctgggcgaagtggccagctttggcggcagcaacatcgagccctctgtgaggagctgcttccagttcgccaacaacaagcccgagatcgaggccgccctgttcctggactggatgaggctggagcctcagagcatggtgtggctgcctgtgctgcacagagtggccgccgccgagaccgccaagcaccaggccaagtgcaatatctgcaaggagtgccccatcatcggcttccggtacaggagcctgaagcacttcaactacgacatctgccagagctgctttttcagcggcagagtggccaagggccacaaaatgcactaccccatggtggagtactgcacccccaccacctccggcgaggatgtgagagacttcgccaaagtgctgaagaataagttccggaccaagcggtactttgccaagcaccccaggatgggctacctgcccgtgcagaccgtgctggaaggcgacaacatggagacctga

SEQ ID NO: 12 - DNA, 8912 bp, synthetic construct
  misc_feature 1..8912: note = Nucleotide sequence of hCK-B84 expression cassette
  source 1..8912: mol_type = other DNA
aattcccatcatcaataatataccttattttggattgaagccaatatgataatgagggggtggagtttgtgacgtggcgcggggcgtgggaacggggcgggtgacgtagtagtctctagaggtccccagcgaccttgacgggcatctgcccggcatttctgacagctttgtgaactgggtggccgagaaggaatgggagttgccgccagattctgacatggatctgaatctgattgagcaggcacccctgaccgtggccgagaagctgcatcgctggcgtaatagcgaagaggcccgcaccgatcgcccttcccaacagttgcgcagcctgaatggcgaatggaattccagacgattgagcgtcaaaatgtaggtatttccatgagcgtttttcctgttgcaatggctggcggtaatattgttctggatattaccagcaaggccgatagtttgagttcttctactcaggcaagtgatgttattactaatcaaagaagtattgcgacaacggttaatttgcgtgatggacagactcttttactcggtggcctcactgattataaaaacacttctcaggattctggcgtaccgttcctgtctaaaatccctttaatcggcctcctgtttagctcccgctctgattctaacgaggaaagcacgttatacgtgctcgtcaaagcaaccatagtacgcgccctgtagcggcgcattaagcgcggcgggtgtggtggttacgcgcagcgtgaccgctacacttgccagcgccctagcgcccgctcctttcgctttcttcccttcctttctcgccacgttcgccggctttccccgtcaagctctaaatcgggggctccctttagggttccgatttagtgctttacggcacctcgaccccaaaaaacttgattagggtgatggttcacgtagtgggccatcgccctgatagacggtttttcgccctttgacgttggagtccacgttctttaatagtggactcttgttccaaactggaacaacactcaaccctatctcggtctattcttttgatttataagggattttgccgatttcggcctattggttaaaaaatgagctgatttaacaaaaatttaacgcgaattttaacaaaatattaacgtttacaatttaaatatttgcttatacaatcttcctgtttttggggcttttctgattatcaaccggggtacatatgattgacatgctagttttacgattaccgttcatcgcctgcaggggggggggggggggggttggccactccctctctgcgcgctcgctcgctcactgaggccgggcgaccaaaggtcgcccgacgcccgggctttgcccgggcggcctcagtgagcgagcgagcgcgcagagagggagtggccaactccatcactaggggttcctagatctgaattcggtaccccactacgggtttaggctgcccatgtaaggaggcaaggcctggggacacccgagatgcctggttataattaacccagacatgtggctgccccccccccccccaacacctgctgcctctaaaaataaccctgtccctggtggatcccctgcatgcgaagatcttcgaacaaggctgtgggggactgagggcaggctgtaacaggcttgggggccagggcttatacgtgcctgggactcccaaagtattactgttccatgttcccggcgaagggccagctgtcccccgccagctagactcagcacttagtttaggaaccagtgagcaagtcagcccttggggcagcccatacaaggccatggggctgggcaagctgcacgcctgggtccggggtgggcacggtgcccgggcaacgagctgaaagctcatctgctctcaggggcccctccctggggacagcccctcctggctagtcacaccctgtaggctcctctatataacccaggggcacaggggctgccctcattctaccaccacctccacagcacagacagacactcaggagccagccagcgtcgagcggccgatccgccaccatgctttggtgggaggaagtggaggactgctacgagagagaggacgtgcagaagaaaaccttcaccaagtgggtgaacgcccagttcagcaagttcggcaagcagcacatcgagaacctgttcagcgacctgcaggatggcaggagactgctggacctgctggagggcctgaccggccagaagctgcccaaggagaagggcagcaccagagtgcacgccctgaacaacgtgaacaaggccctgagagtgctgcagaacaacaacgtggacctggtgaacatcggcagcaccgacatcgtggacggcaaccacaagctgaccctgggcctgatctggaacatcatcctgcactggcaggtgaagaacgtgatgaagaacatcatggccggcctgcagcagaccaacagcgagaagatcctgctgagctgggtgaggcagagcaccagaaactacccccaggtgaacgtgatcaacttcaccacctcctggagcgacggcctggccctgaacgccctgatccacagccacagacccgacctgttcgactggaacagcgtggtgtgtcagcagagcgccacccagagactggagcacgccttcaacatcgccagataccagctgggcatcgagaagctgctggaccccgaggacgtggacaccacctaccccgacaagaaaagcatcctcatgtacattaccagcctgttccaggtgctgccccagcaggtgtccatcgaggccatccaggaagtggaaatgctgcccaggccccccaaagtgaccaaggaggagcacttccagctgcaccaccagatgcactacagccagcagatcacagtgagcctggcccagggctatgagagaaccagcagccccaagcccagattcaagagctacgcctacacccaggccgcctacgtgaccacctccgaccccaccagaagccccttccccagccagcacctggaggcccccgaggacaagagcttcggcagcagcctgatggagagcgaagtgaacctggacagataccagaccgccctggaggaagtgctgtcctggctgctgagcgccgaggacaccctgcaggcccagggcgagatcagcaacgacgtggaagtggtgaaggaccagttccacacccacgagggctacatgatggatctgaccgcccaccagggcagagtgggcaatatcctgcagctgggcagcaagctgatcggcaccggcaagctgagcgaggacgaggagaccgaagtgcaggagcagatgaacctgctgaacagcagatgggagtgcctgagagtggccagcatggagaagcagagcaacctgcacagagtgctgatggacctgcagaaccagaagctgaaggagctgaacgactggctgaccaagaccgaggagcggaccagaaagatggaggaggagcccctgggccccgacctggaggacctgaagagacaggtgcagcagcacaaagtgctgcaggaggacctggagcaggagcaggtgcgcgtgaacagcctgacccacatggtggtggtcgtggacgagagcagcggcgaccacgccacagccgccctggaagagcagctgaaagtgctgggcgacagatgggccaatatttgtaggtggaccgaggacagatgggtgctgctgcaggaccagcccgacctggcccctggcctgaccaccatcggcgccagccccacccagaccgtgaccctggtgacccagcccgtggtgacaaaggagaccgccatcagcaagctggagatgcccagctccctgatgctggaagtgcccacccaccgcctgctccagcagttccccctggacctggagaagttcctggcctggctgaccgaggccgaaaccaccgccaatgtgctccaggacgccactagaaaggagaggctgctggaggacagcaagggcgtgaaagagctgatgaagcagtggcaggatctgcagggcgaaatcgaggcccacaccgacgtgtaccacaacctggacgagaacagccagaagattctgaggagcctggagggcagcgacgacgccgtcctgctccagaggaggctggacaacatgaacttcaagtggagcgagctgcggaagaagagcctgaacatccggagccacctggaagccagcagcgaccagtggaagagactgcacctgagcctgcaggagctgctggtgtggctgcagctgaaggacgacgagctgagcagacaggcccccatcggcggcgacttccccgccgtgcagaagcagaacgacgtgcaccgggccttcaagagggagctgaaaaccaaggaacccgtgatcatgagcaccctggagacagtgcggatcttcctgaccgagcagcccctggagggactggagaagctgtaccaggagcccagagagctgccccccgaggagagagcccagaacgtgaccaggctgctgagaaagcaggccgaggaagtgaataccgagtgggagaagctgaatctgcacagcgccgactggcagagaaagatcgacgagaccctggagagactccaggaactgcaggaagccaccgacgagctggacctgaagctgagacaggccgaagtgatcaagggcagctggcagcctgtgggcgatctgctgatcgactccctgcaggatcacctggagaaagtgaaggccctgcggggcgagatcgcccccctgaaggagaatgtgagccacgtgaacgacctggccagacagctgaccaccctgggcatccagctgagcccctacaacctgagcacactggaggatctgaacacccggtggaaactgctgcaggtggccgtggaggatagagtgaggcagctgcacgaagcccacagagacttcggccctgcctcccagcacttcctgagcaccagcgtgcagggcccctgggagagagccatctcccccaacaaagtgccctactacatcaaccacgagacccagaccacctgctgggaccaccctaagatgaccgagctgtatcagagcctggccgacctgaacaatgtgcggttcagcgcctacagaaccgccatgaagctgcggagactgcagaaggccctgtgcctggatctgctgagcctgagcgccgcctgcgacgccctggaccagcacaacctgaagcagaatgaccagcccatggacatcctgcagatcatcaactgcctgaccacaatctacgaccggctggaacaggagcacaacaacctggtgaatgtgcccctgtgcgtggacatgtgcctgaattggctgctgaacgtgtacgacaccggcaggaccggcagaatccgcgtgctgagcttcaagaccggcatcatcagcctgtgcaaggcccacctggaggataagtaccgctacctgttcaagcaggtggccagcagcaccggcttctgcgatcagaggagactgggcctgctgctgcacgatagcatccagatccctaggcagctgggcgaagtggccagctttggcggcagcaacatcgagccctctgtgaggagctgcttccagttcgccaacaacaagcccgagatcgaggccgccctgttcctggactggatgaggctggagcctcagagcatggtgtggctgcctgtgctgcacagagtggccgccgccgagaccgccaagcaccaggccaagtgcaatatctgcaaggagtgccccatcatcggcttccggtacaggagcctgaagcacttcaactacgacatctgccagagctgctttttcagcggcagagtggccaagggccacaaaatgcactaccccatggtggagtactgcacccccaccacctccggcgaggatgtgagagacttcgccaaagtgctgaagaataagttccggaccaagcggtactttgccaagcaccccaggatgggctacctgcccgtgcagaccgtgctggaaggcgacaacatggagacctgatgaggagctcgagaggcctaataaagagctcagatgcatcgatcagagtgtgttggttttttgtgtgagatctaggaacccctagtgatggagttggccactccctctctgcgcgctcgctcgctcactgaggccgcccgggcaaagcccgggcgtcgggcgacctttggtcgcccggcctcagtgagcgagcgagcgcgcagagagggagtggccaacccccccccccccccccctgcaggcgattctcttgtttgctccagactctcaggcaatgacctgatagcctttgtagagacctctcaaaaatagctaccctctccggcatgaatttatcagctagaacggttgaatatcatattgatggtgatttgactgtctccggcctttctcacccgtttgaatctttacctacacattactcaggcattgcatttaaaatatatgagggttctaaaaatttttatccttgcgttgaaataaaggcttctcccgcaaaagtattacagggtcataatgtttttggtacaaccgatttagctttatgctctgaggctttattgcttaattttgctaattctttgccttgcctgtatgatttattggatgttggaattcctgatgcggtattttctccttacgcatctgtgcggtatttcacaccgcatatggtgcactctcagtacaatctgctctgatgccgcatagttaagccagccccgacacccgccaacacccgctgacgcgccctgacgggcttgtctgctcccggcatccgcttacagacaagctgtgaccgtctccgggagctgcatgtgtcagaggttttcaccgtcatcaccgaaacgcgcgagacgaaagggcctcgtgatacgcctatttttataggttaatgtcatgataataatggtttcttagacgtcaggtggcacttttcggggaaatgtgcgcggaacccctatttgtttatttttctaaatacattcaaatatgtatccgctcatgagacaataaccctgataaatgcttcaataatattgaaaaaggaagagtatgagtattcaacatttccgtgtcgcccttattcccttttttgcggcattttgccttcctgtttttgctcacccagaaacgctggtgaaagtaaaagatgctgaagatcagttgggtgcacgagtgggttacatcgaactggatctcaacagcggtaagatccttgagagttttcgccccgaagaacgttttccaatgatgagcacttttaaagttctgctatgtggcgcggtattatcccgtattgacgccgggcaagagcaactcggtcgccgcatacactattctcagaatgacttggttgagtactcaccagtcacagaaaagcatcttacggatggcatgacagtaagagaattatgcagtgctgccataaccatgagtgataacactgcggccaacttacttctgacaacgatcggaggaccgaaggagctaaccgcttttttgcacaacatgggggatcatgtaactcgccttgatcgttgggaaccggagctgaatgaagccataccaaacgacgagcgtgacaccacgatgcctgtagcaatggcaacaacgttgcgcaaactattaactggcgaactacttactctagcttcccggcaacaattaatagactggatggaggcggataaagttgcaggaccacttctgcgctcggcccttccggctggctggtttattgctgataaatctggagccggtgagcgtgggtctcgcggtatcattgcagcactggggccagatggtaagccctcccgtatcgtagttatctacacgacggggagtcaggcaactatggatgaacgaaatagacagatcgctgagataggtgcctcactgattaagcattggtaactgtcagaccaagtttactcatatatactttagattgatttaaaacttcatttttaatttaaaaggatctaggtgaagatcctttttgataatctcatgaccaaaatcccttaacgtgagttttcgttccactgagcgtcagaccccgtagaaaagatcaaaggatcttcttgagatcctttttttctgcgcgtaatctgctgcttgcaaacaaaaaaaccaccgctaccagcggtggtttgtttgccggatcaagagctaccaactctttttccgaaggtaactggcttcagcagagcgcagataccaaatactgtccttctagtgtagccgtagttaggccaccacttcaagaactctgtagcaccgcctacatacctcgctctgctaatcctgttaccagtggctgctgccagtggcgataagtcgtgtcttaccgggttggactcaagacgatagttaccggataaggcgcagcggtcgggctgaacggggggttcgtgcacacagcccagcttggagcgaacgacctacaccgaactgagatacctacagcgtgagctatgagaaagcgccacgcttcccgaagggagaaaggcggacaggtatccggtaagcggcagggtcggaacaggagagcgcacgagggagcttccagggggaaacgcctggtatctttatagtcctgtcgggtttcgccacctctgacttgagcgtcgatttttgtgatgctcgtcaggggggcggagcctatggaaaaacgccagcaacgcggcctttttacggttcctggccttttgctggccttttgctcacatgttctttcctgcgttatcccctgattctgtggataaccgtattaccgcctttgagtgagctgataccgctcgccgcagccgaacgaccgagcgcagcgagtcagtgagcgaggaagcggaagagcgcccaatacgcaaaccgcctctccccgcgcgttggccgattcattaatgcag

SEQ ID NO: 13 - protein, 1325 aa, synthetic construct
  REGION 1..1325: note = Protein product of hCK-B84 expression cassette
MLWWEEVEDCYEREDVQKKTFTKWVNAQFSKFGKQHIENLFSDLQDGRRLLDLLEGLTGQKLPKEKGSTRVHALNNVNKALRVLQNNNVDLVNIGSTDIVDGNHKLTLGLIWNIILHWQVKNVMKNIMAGLQQTNSEKILLSWVRQSTRNYPQVNVINFTTSWSDGLALNALIHSHRPDLFDWNSVVCQQSATQRLEHAFNIARYQLGIEKLLDPEDVDTTYPDKKSILMYITSLFQVLPQQVSIEAIQEVEMLPRPPKVTKEEHFQLHHQMHYSQQITVSLAQGYERTSSPKPRFKSYAYTQAAYVTTSDPTRSPFPSQHLEAPEDKSFGSSLMESEVNLDRYQTALEEVLSWLLSAEDTLQAQGEISNDVEVVKDQFHTHEGYMMDLTAHQGRVGNILQLGSKLIGTGKLSEDEETEVQEQMNLLNSRWECLRVASMEKQSNLHRVLMDLQNQKLKELNDWLTKTEERTRKMEEEPLGPDLEDLKRQVQQHKVLQEDLEQEQVRVNSLTHMVVVVDESSGDHATAALEEQLKVLGDRWANICRWTEDRWVLLQDQPDLAPGLTTIGASPTQTVTLVTQPVVTKETAISKLEMPSSLMLEVPTHRLLQQFPLDLEKFLAWLTEAETTANVLQDATRKERLLEDSKGVKELMKQWQDLQGEIEAHTDVYHNLDENSQKILRSLEGSDDAVLLQRRLDNMNFKWSELRKKSLNIRSHLEASSDQWKRLHLSLQELLVWLQLKDDELSRQAPIGGDFPAVQKQNDVHRAFKRELKTKEPVIMSTLETVRIFLTEQPLEGLEKLYQEPRELPPEERAQNVTRLLRKQAEEVNTEWEKLNLHSADWQRKIDETLERLQELQEATDELDLKLRQAEVIKGSWQPVGDLLIDSLQDHLEKVKALRGEIAPLKENVSHVNDLARQLTTLGIQLSPYNLSTLEDLNTRWKLLQVAVEDRVRQLHEAHRDFGPASQHFLSTSVQGPWERAISPNKVPYYINHETQTTCWDHPKMTELYQSLADLNNVRFSAYRTAMKLRRLQKALCLDLLSLSAACDALDQHNLKQNDQPMDILQIINCLTTIYDRLEQEHNNLVNVPLCVDMCLNWLLNVYDTGRTGRIRVLSFKTGIISLCKAHLEDKYRYLFKQVASSTGFCDQRRLGLLLHDSIQIPRQLGEVASFGGSNIEPSVRSCFQFANNKPEIEAALFLDWMRLEPQSMVWLPVLHRVAAAETAKHQAKCNICKECPIIGFRYRSLKHFNYDICQSCFFSGRVAKGHKMHYPMVEYCTPTTSGEDVRDFAKVLKNKFRTKRYFAKHPRMGYLPVQTVLEGDNMET